European Patent Specification EP 3 510 187 B1, published September 6, 2023. Title: Antobody library. Applicant: Italfarmaco. The sequence listing filed with the application follows.

SEQUENCE LISTING (11 sequences)

SEQ ID NO: 1 - protein, 97 aa, Homo sapiens
  Heavy chain VH3 translated germline segment V3-23
EVQLLESGGGLVQPGGSLRLSCAASGFTFSSYAMSWVRQAPGKGLEWVSAISGSGGSTYYADSVKGRFTISRDNSKNTLYLQMNSLRAEDTAVYYCA

SEQ ID NO: 2 - protein, 11 aa, Homo sapiens
  Heavy chain translated J4 germline segment
WGQGTLVTVSS

SEQ ID NO: 3 - protein, 88 aa, Homo sapiens
  Kappa light chain VK1 translated germline segment
DIQMTQSPSSLSASVGDRVTITCRASQSISSYLNWYQQKPGKAPKLLIYAASSLQSGVPSRFSGSGSGTDFTLTISSLQPEDFATYYC

SEQ ID NO: 4 - protein, 11 aa, Homo sapiens
  Kappa light chain VK1 translated germline segment J1
FGQGTKVEIKR

SEQ ID NO: 5 - protein, 9 aa, Homo sapiens
  Kappa light chain CDR3
QQSYSTPLT

SEQ ID NO: 6 - protein, 15 aa, Homo sapiens
  VH/VL linker
GGGGSGGGGSGGGGS

SEQ ID NO: 7 - DNA, 1032 bp, Homo sapiens
  source 1..1032: /mol_type="unassigned DNA" /note="Scaffold including stuffer" /organism="Homo sapiens"
gaagttcagctgctggaatctggtggtggtctggttcagccgggtggttctctgcgtctgtcttgcgctgcttctggtttcaccttctcttcttacgctatgtcttgggttcgtcaggctccgggtaaaggtctggaatgggtttctgctatctctggttctggtggttctacctactacgctgactctgttaaaggtcgtttcaccatctctcgtgacaactctaaaaacaccctgtacctgcaaatgaactctctgcgtgctgaagacactgcagggcactaaatatgtaacacactcaatatcaacatgacctcaaacacaggctcttacaaaggtagaagaaattttagttatggaaaattgagctatgctaattgttcccatagtggaagtttgaactgaagtcgtgcgcagaacatcaagggcagtagaaactttctatatcacgcaaggacatcgatatcgaagcccgtaccgtgagaactttttcagtacggcaaagtatactaggcctattgcccttttcgtaacttgtgcgtattctctttcatcactgttcacaaccagtaccttgtcctcaaaaggtcatcacgtttatttaaattcccattcgaaaggcatacatcgtagtgccaaggcacactcgttaccgtctcaagtggtggcggaggatccggaggaggtggctctggaggtggcggttcagacatccagatgacccagtctccgtcttctctgtctgctagcgttggcgatcgtgttaccatcacctgccgtgcttctcagtctatctcttcttacctgaactggtatcagcagaaacccgggaaagctccgaaactgctgatctacgctgcttcttctcttcagtctggtgttccgtctcgtttctctggttctggttctggcaccgacttcaccctgaccatctcgagccttcagccggaagacttcgctacctactactgccagcagtcttactctaccccgctgaccttcggtcagggtaccaaagttgaaatcaaacgt

SEQ ID NO: 8 - DNA, 5540 bp, Homo sapiens
  source 1..5540: /mol_type="other DNA" /note="Base vector VH3_VK1_v22" /organism="Homo sapiens"
gacgaaagggcctcgtgatacgcctatttttataggttaatgtcatgataataatggtttcttagacgtcaggtggcacttttcggggaaatgtgcgcggaacccctatttgtttatttttctaaatacattcaaatatgtatccgctcatgagacaataaccctgataaatgcttcaataatattgaaaaaggaagagtatgagtattcaacatttccgtgtcgcccttattcccttttttgcggcattttgccttcctgtttttgctcacccagaaacgctggtgaaagtaaaagatgctgaagatcagttgggtgcccgagtgggttacatcgaactggatctcaacagcggtaagatccttgagagttttcgccccgaagaacgttttccaatgatgagcacttttaaagttctgctatgtggcgcggtattatcccgtattgacgccgggcaagagcaactcggtcgccgcatacactattctcagaatgacttggttgagtactcaccagtcacagaaaagcatcttacggatggcatgacagtaagagaattatgcagtgctgccataaccatgagtgataacactgcggccaacttacttctgacaaccatcggaggaccgaaggagctaaccgcttttttgcacaacatgggggatcatgtaactcgccttgatcgttgggaaccggagctgaatgaagccataccaaacgacgagcgtgacaccacgatgcctgtagcaatggcaacaacgttgcgcaaactattaactggcgaactacttactctagcttcccggcaacaattaatagactggatggaggcggataaagttgcaggaccacttctgcgctcggcccttccggctggctggtttattgctgataaatctggagccggtgagcgtgggtctcgcggtatcattgcagcactggggccagatggtaagccctcccgtatcgtagttatctacacgacggggagtcaggcaactatggatgaacgaaatagacagatcgctgagataggtgcctcactgattaagcattggtaactgtcagaccaagtttactcatatatactttagattgatttaaaacttcatttttaatttaaaaggatctaggtgaagatcctttttgataatctcatgaccaaaatcccttaacgtgagttttcgttccactgagcgtcagaccccgtagaaaagatcaaaggatcttcttgagatcctttttttctgcgcgtaatctgctgcttgcaaacaaaaaaaccaccgctaccagcggtggtttgtttgccggatcaagagctaccaactctttttccgaaggtaactggcttcagcagagcgcagataccaaatactgtccttctagtgtagccgtagttaggccaccacttcaagaactctgtagcaccgcctacatacctcgctctgctaatcctgttaccagtggctgctgccagtggcgataagtcgtgtcttaccgggttggactcaagacgatagttaccggataaggcgcagcggtcgggctgaacggggggttcgtgcatacagcccagcttggagcgaacgacctacaccgaactgagatacctacagcgtgagcattgagaaagcgccacgcttcccgaagggagaaaggcggacaggtatccggtaagcggcagggtcggaacaggagagcgcacgagggagcttccagggggaaacgcctggtatctttatagtcctgtcgggtttcgccacctctgacttgagcgtcgatttttgtgatgctcgtcaggggggcggagcctatggaaaaacgccagcaacgcggcctttttacggttcctggccttttgctggccttttgctcacatgttctttcctgcgttatcccctgattctgtggataaccgtattaccgcctttgagtgagctgataccgctcgccgcagccgaacgaccgagcgcagcgagtcagtgagcgaggaagcggaagagcgcccaatacgcaaaccgcctctccccgcgcgttggccgattcattaatgcagctggcacgacaggtttcccgactggaaagcgggcagtgagcgcaacgcaattaatgtgagttagctcactcattaggcaccccaggctttacactttatgcttccggctcgtatgttgtgtggaattgtgagcggataacaatttcacacaggaaacagctatgaccatgattacgccaagctttggagccttttttttggagattttcaacgtgaaaaaattattattcgcaattcctttagttgttcctttctatgcggcccagccggcgatggccgaagttcagctgctggaatctggtggtggtctggttcagccgggtggttctctgcgtctgtcttgcgctgcttctggtttcaccttctcttcttacgctatgtcttgggttcgtcaggctccgggtaaaggtctggaatgggtttctgctatctctggttctggtggttctacctactacgctgactctgttaaaggtcgtttcaccatctctcgtgacaactctaaaaacaccctgtacctgcaaatgaactctctgcgtgctgaagacactgcagggcactaaatatgtaacacactcaatatcaacatgacctcaaacacaggctcttacaaaggtagaagaaattttagttatggaaaattgagctatgctaattgttcccatagtggaagtttgaactgaagtcgtgcgcagaacatcaagggcagtagaaactttctatatcacgcaaggacatcgatatcgaagcccgtaccgtgagaactttttcagtacggcaaagtatactaggcctattgcccttttcgtaacttgtgcgtattctctttcatcactgttcacaaccagtaccttgtcctcaaaaggtcatcacgtttatttaaattcccattcgaaaggcatacatcgtagtgccaaggcacactcgttaccgtctcaagtggtggcggaggatccggaggaggtggctctggaggtggcggttcagacatccagatgacccagtctccgtcttctctgtctgctagcgttggcgatcgtgttaccatcacctgccgtgcttctcagtctatctcttcttacctgaactggtatcagcagaaacccgggaaagctccgaaactgctgatctacgctgcttcttctcttcagtctggtgttccgtctcgtttctctggttctggttctggcaccgacttcaccctgaccatctcgagccttcagccggaagacttcgctacctactactgccagcagtcttactctaccccgctgaccttcggtcagggtaccaaagttgaaatcaaacgtgcggccgcacatcatcatcaccatcacggggccgcagaacaaaaactcatctcagaagaggatctgaatggggccgcatagactgttgaaagttgtttagcaaaacctcatacagaaaattcatttactaacgtctggaaagacgacaaaactttagatcgttacgctaactatgagggctgtctgtggaatgctacaggcgttgtggtttgtactggtgacgaaactcagtgttacggtacatgggttcctattgggcttgctatccctgaaaatgagggtggtggctctgagggtggcggttctgagggtggcggttctgagggtggcggtactaaacctcctgagtacggtgatacacctattccgggctatacttatatcaaccctctcgacggcacttatccgcctggtactgagcaaaaccccgctaatcctaatccttctcttgaggagtctcagcctcttaatactttcatgtttcagaataataggttccgaaataggcagggtgcattaactgtttatacgggcactgttactcaaggcactgaccccgttaaaacttattaccagtacactcctgtatcatcaaaagccatgtatgacgcttactggaacggtaaattcagagactgcgctttccattctggctttaatgaagatccattcgtttgtgaatatcaaggccaatcgtctgacctgcctcaacctcctgtcaatgctggcggcggctctggtggtggttctggtggcggctctgagggtggcggctctgagggtggcggttctgagggtggcggctctgagggtggcggttccggtggcggctccggttccggtgattttgattatgaaaaaatggcaaacgctaataagggggctatgaccgaaaatgccgatgaaaacgcgctacagtctgacgctaaaggcaaacttgattctgtcgctactgattacggtgctgctatcgatggtttcattggtgacgtttccggccttgctaatggtaatggtgctactggtgattttgctggctctaattcccaaatggctcaagtcggtgacggtgataattcacctttaatgaataatttccgtcaatatttaccttctttgcctcagtcggttgaatgtcgcccttatgtctttggcgctggtaaaccatatgaattttctattgattgtgacaaaataaacttattccgtggtgtctttgcgtttcttttatatgttgccacctttatgtatgtattttcgacgtttgctaacatactgcgtaataaggagtcttaataagaattcactggccgtcgttttacaacgtcgtgactgggaaaaccctggcgttacccaacttaatcgccttgcagcacatccccctttcgccagctggcgtaatagcgaagaggcccgcaccgctcgcccttcccaacagttgcgcagcctgaatggcgaatggcgcctgatgcggtattttctccttacgcatctgtgcggtatttcacaccgcatataaattgtaaacgttaatattttgttaaaattcgcgttaaatttttgttaaatcagctcattttttaaccaataggccgaaatcggcaaaatcccttataaatcaaaagaatagcccgagatagggttgagtgttgttccagtttggaacaagagtccactattaaagaacgtggactccaacgtcaaagggcgaaaaaccgtctatcagggcgatggcccactacgtgaaccatcacccaaatcaagttttttggggtcgaggtgccgtaaagcactaaatcggaaccctaaagggagcccccgatttagagcttgacggggaaagccggcgaacgtggcgagaaaggaagggaagaaagcgaaaggagcgggcgctagggcgctggcaagtgtagcggtcacgctgcgcgtaaccaccacacccgccgcgcttaatgcgccgctacagggcgcgtactatggttgctttgacgggtgcagtctcagtacaatctgctctgatgccgcatagttaagccagccccgacacccgccaacacccgctgacgcgccctgacgggcttgtctgctcccggcatccgcttacagacaagctgtgaccgtctccgggagctgcatgtgtcagaggttttcaccgtcatcaccgaaacgcgcga

SEQ ID NO: 9 - DNA, 15 bp, Homo sapiens
  source 1..15: /mol_type="other DNA" /note="Sty_rev_1" /organism="Homo sapiens"
ccgaccttggcccca

SEQ ID NO: 10 - DNA, 27 bp, Homo sapiens
  source 1..27: /mol_type="other DNA" /note="PstI_for _1 primer" /organism="Homo sapiens"
cgaaaagcacctgcagtgtattactgc

SEQ ID NO: 11 - DNA, 19 bp, Homo sapiens
  source 1..19: /mol_type="other DNA" /note="Sty_rev_2 primer" /organism="Homo sapiens"
ctgaccgacctgggcccca